European Patent Application EP 4 295 857 A1, published December 27, 2023. Title: Pharmaceutical compositions for preventing or treating fibrotic diseases comprising progranulin or active fragments thereof as an active ingredient. Applicant: THE ASAN FOUNDATION University of Ulsan Foundation For Industry Cooperation. The sequence listing filed with the application follows.

SEQUENCE LISTING (14 sequences)

SEQ ID NO: 1 - protein, 54 aa, Artificial Sequence
  C-granule in hPGRN
VPCDNVSSCPSSDTCCQLTSGEWGCCPIPEAVCCSDHQHCCPQGYTCVAEGQCQ

SEQ ID NO: 2 - protein, 333 aa, Artificial Sequence
  hPGRN-FBAC
GHHCCPRGFHCSADGRSCFQRSGNNSVGAIQCPDSQFECPDFSTCCVMVDGSWGCCPMPQASCCEDRVHCCPHGAFCDLVHTRCITPTGTHPLAKKLPAQRTNRAVALSSSVMCPDARSRCPDGSTCCELPSGKYGCCPMPNATCCSDHLHCCPQDTVCDLIQSKCLSKENATTDLLTKLPAHTVGDVKCDMEVSCPDGYTCCRLQSGAWGCCPFTQAVCCEDHIHCCPAGFTCDTQKGTCEQGPHQVPWMEKAPAHLSLPDPQALKRDVPCDNVSSCPSSDTCCQLTSGEWGCCPIPEAVCCSDHQHCCPQGYTCVAEGQCQRGSEIVAGLE

SEQ ID NO: 3 - protein, 305 aa, Artificial Sequence
  hPGRN-BACD
ALSSSVMCPDARSRCPDGSTCCELPSGKYGCCPMPNATCCSDHLHCCPQDTVCDLIQSKCLSKENATTDLLTKLPAHTVGDVKCDMEVSCPDGYTCCRLQSGAWGCCPFTQAVCCEDHIHCCPAGFTCDTQKGTCEQGPHQVPWMEKAPAHLSLPDPQALKRDVPCDNVSSCPSSDTCCQLTSGEWGCCPIPEAVCCSDHQHCCPQGYTCVAEGQCQRGSEIVAGLEKMPARRASLSHPRDIGCDQHTSCPVGQTCCPSLGGSWACCQLPHAVCCEDRQHCCPAGYTCNVKARSCEKEVVSAQPA

SEQ ID NO: 4 - protein, 242 aa, Artificial Sequence
  hPGRN-CDE
LSLPDPQALKRDVPCDNVSSCPSSDTCCQLTSGEWGCCPIPEAVCCSDHQHCCPQGYTCVAEGQCQRGSEIVAGLEKMPARRASLSHPRDIGCDQHTSCPVGQTCCPSLGGSWACCQLPHAVCCEDRQHCCPAGYTCNVKARSCEKEVVSAQPATFLARSPHVGVKDVECGEGHFCHDNQTCCRDNRQGWACCPYRQGVCCADRRHCCPAGFRCAARGTKCLRREAPRWDAPLRDPALRQLL

SEQ ID NO: 5 - protein, 593 aa, Artificial Sequence
  full length hPGRN
MWTLVSWVALTAGLVAGTRCPDGQFCPVACCLDPGGASYSCCRPLLDKWPTTLSRHLGGPCQVDAHCSAGHSCIFTVSGTSSCCPFPEAVACGDGHHCCPRGFHCSADGRSCFQRSGNNSVGAIQCPDSQFECPDFSTCCVMVDGSWGCCPMPQASCCEDRVHCCPHGAFCDLVHTRCITPTGTHPLAKKLPAQRTNRAVALSSSVMCPDARSRCPDGSTCCELPSGKYGCCPMPNATCCSDHLHCCPQDTVCDLIQSKCLSKENATTDLLTKLPAHTVGDVKCDMEVSCPDGYTCCRLQSGAWGCCPFTQAVCCEDHIHCCPAGFTCDTQKGTCEQGPHQVPWMEKAPAHLSLPDPQALKRDVPCDNVSSCPSSDTCCQLTSGEWGCCPIPEAVCCSDHQHCCPQGYTCVAEGQCQRGSEIVAGLEKMPARRASLSHPRDIGCDQHTSCPVGQTCCPSLGGSWACCQLPHAVCCEDRQHCCPAGYTCNVKARSCEKEVVSAQPATFLARSPHVGVKDVECGEGHFCHDNQTCCRDNRQGWACCPYRQGVCCADRRHCCPAGFRCAARGTKCLRREAPRWDAPLRDPALRQLL

SEQ ID NO: 6 - DNA, 162 bp, Artificial Sequence
  C-granule in hPGRN
gtcccctgtgataatgtcagcagctgtccctcctccgatacctgctgccaactcacgtctggggagtggggctgctgtccaatcccagaggctgtctgctgctcggaccaccagcactgctgcccccagggctacacgtgtgtagctgaggggcagtgtcag

SEQ ID NO: 7 - DNA, 999 bp, Artificial Sequence
  hPGRN-FBAC
ggccatcactgctgcccacggggcttccactgcagtgcagacgggcgatcctgcttccaaagatcaggtaacaactccgtgggtgccatccagtgccctgatagtcagttcgaatgcccggacttctccacgtgctgtgttatggtcgatggctcctgggggtgctgccccatgccccaggcttcctgctgtgaagacagggtgcactgctgtccgcacggtgccttctgcgacctggttcacacccgctgcatcacacccacgggcacccaccccctggcaaagaagctccctgcccagaggactaacagggcagtggccttgtccagctcggtcatgtgtccggacgcacggtcccggtgccctgatggttctacctgctgtgagctgcccagtgggaagtatggctgctgcccaatgcccaacgccacctgctgctccgatcacctgcactgctgcccccaagacactgtgtgtgacctgatccagagtaagtgcctctccaaggagaacgctaccacggacctcctcactaagctgcctgcgcacacagtgggggatgtgaaatgtgacatggaggtgagctgcccagatggctatacctgctgccgtctacagtcgggggcctggggctgctgcccttttacccaggctgtgtgctgtgaggaccacatacactgctgtcccgcggggtttacgtgtgacacgcagaagggtacctgtgaacaggggccccaccaggtgccctggatggagaaggccccagctcacctcagcctgccagacccacaagccttgaagagagatgtcccctgtgataatgtcagcagctgtccctcctccgatacctgctgccaactcacgtctggggagtggggctgctgtccaatcccagaggctgtctgctgctcggaccaccagcactgctgcccccagggctacacgtgtgtagctgaggggcagtgtcagcgaggaagcgagatcgtggctggactggag

SEQ ID NO: 8 - DNA, 915 bp, Artificial Sequence
  hPGRN-BACD
gccttgtccagctcggtcatgtgtccggacgcacggtcccggtgccctgatggttctacctgctgtgagctgcccagtgggaagtatggctgctgcccaatgcccaacgccacctgctgctccgatcacctgcactgctgcccccaagacactgtgtgtgacctgatccagagtaagtgcctctccaaggagaacgctaccacggacctcctcactaagctgcctgcgcacacagtgggggatgtgaaatgtgacatggaggtgagctgcccagatggctatacctgctgccgtctacagtcgggggcctggggctgctgcccttttacccaggctgtgtgctgtgaggaccacatacactgctgtcccgcggggtttacgtgtgacacgcagaagggtacctgtgaacaggggccccaccaggtgccctggatggagaaggccccagctcacctcagcctgccagacccacaagccttgaagagagatgtcccctgtgataatgtcagcagctgtccctcctccgatacctgctgccaactcacgtctggggagtggggctgctgtccaatcccagaggctgtctgctgctcggaccaccagcactgctgcccccagggctacacgtgtgtagctgaggggcagtgtcagcgaggaagcgagatcgtggctggactggagaagatgcctgcccgccgggcttccttatcccaccccagagacatcggctgtgaccagcacaccagctgcccggtggggcagacctgctgcccgagcctgggtgggagctgggcctgctgccagttgccccatgctgtgtgctgcgaggatcgccagcactgctgcccggctggctacacctgcaacgtgaaggctcgatcctgcgagaaggaagtggtctctgcccagcctgcc

SEQ ID NO: 9 - DNA, 726 bp, Artificial Sequence
  hPGRN-CDE
ctcagcctgccagacccacaagccttgaagagagatgtcccctgtgataatgtcagcagctgtccctcctccgatacctgctgccaactcacgtctggggagtggggctgctgtccaatcccagaggctgtctgctgctcggaccaccagcactgctgcccccagggctacacgtgtgtagctgaggggcagtgtcagcgaggaagcgagatcgtggctggactggagaagatgcctgcccgccgggcttccttatcccaccccagagacatcggctgtgaccagcacaccagctgcccggtggggcagacctgctgcccgagcctgggtgggagctgggcctgctgccagttgccccatgctgtgtgctgcgaggatcgccagcactgctgcccggctggctacacctgcaacgtgaaggctcgatcctgcgagaaggaagtggtctctgcccagcctgccaccttcctggcccgtagccctcacgtgggtgtgaaggacgtggagtgtggggaaggacacttctgccatgataaccagacctgctgccgagacaaccgacagggctgggcctgctgtccctaccgccagggcgtctgttgtgctgatcggcgccactgctgtcctgctggcttccgctgcgcagccaggggtaccaagtgtttgcgcagggaggccccgcgctgggacgcccctttgagggacccagccttgagacagctgctg

SEQ ID NO: 10 - DNA, 1761 bp, Artificial Sequence
  full length hPGRN
acgcggtgcccagatggtcagttctgccctgtggcctgctgcctggaccccggaggagccagctacagctgctgccgtccccttctggacaaatggcccacaacactgagcaggcatctgggtggcccctgccaggttgatgcccactgctctgccggccactcctgcatctttaccgtctcagggacttccagttgctgccccttcccagaggccgtggcatgcggggatggccatcactgctgcccacggggcttccactgcagtgcagacgggcgatcctgcttccaaagatcaggtaacaactccgtgggtgccatccagtgccctgatagtcagttcgaatgcccggacttctccacgtgctgtgttatggtcgatggctcctgggggtgctgccccatgccccaggcttcctgctgtgaagacagggtgcactgctgtccgcacggtgccttctgcgacctggttcacacccgctgcatcacacccacgggcacccaccccctggcaaagaagctccctgcccagaggactaacagggcagtggccttgtccagctcggtcatgtgtccggacgcacggtcccggtgccctgatggttctacctgctgtgagctgcccagtgggaagtatggctgctgcccaatgcccaacgccacctgctgctccgatcacctgcactgctgcccccaagacactgtgtgtgacctgatccagagtaagtgcctctccaaggagaacgctaccacggacctcctcactaagctgcctgcgcacacagtgggggatgtgaaatgtgacatggaggtgagctgcccagatggctatacctgctgccgtctacagtcgggggcctggggctgctgcccttttacccaggctgtgtgctgtgaggaccacatacactgctgtcccgcggggtttacgtgtgacacgcagaagggtacctgtgaacaggggccccaccaggtgccctggatggagaaggccccagctcacctcagcctgccagacccacaagccttgaagagagatgtcccctgtgataatgtcagcagctgtccctcctccgatacctgctgccaactcacgtctggggagtggggctgctgtccaatcccagaggctgtctgctgctcggaccaccagcactgctgcccccagggctacacgtgtgtagctgaggggcagtgtcagcgaggaagcgagatcgtggctggactggagaagatgcctgcccgccgggcttccttatcccaccccagagacatcggctgtgaccagcacaccagctgcccggtggggcagacctgctgcccgagcctgggtgggagctgggcctgctgccagttgccccatgctgtgtgctgcgaggatcgccagcactgctgcccggctggctacacctgcaacgtgaaggctcgatcctgcgagaaggaagtggtctctgcccagcctgccaccttcctggcccgtagccctcacgtgggtgtgaaggacgtggagtgtggggaaggacacttctgccatgataaccagacctgctgccgagacaaccgacagggctgggcctgctgtccctaccgccagggcgtctgttgtgctgatcggcgccactgctgtcctgctggcttccgctgcgcagccaggggtaccaagtgtttgcgcagggaggccccgcgctgggacgcccctttgagggacccagccttgagacagctgctgtgcccaactttcttgtacaaagtggttgatatc

SEQ ID NO: 11 - DNA, 4734 bp, Artificial Sequence
  pPM-C-His
ttttggattgaagccaatatgataatgagggggtggagtttgtgacgtggcgcggggcgtgggaacggggcgggtgacgtagtagtgtggcggaagtgtgatgttgcaagtgtggcggaacacatgtaagcgacggatgtggcaaaagtgacgtttttggtgtgcgccggtgtacacaggaagtgacaattttcgcgcggttttaggcggatgttgtagtaaatttgggcgtaaccgagtaagatttggccattttcgcgggaaaactgaataagaggaagtgaaatctgaataattttgtgttactcatagcgcgtaatacggcagacctcagcgctagattattgaagcatttatcagggttattgtctcatgagcggatacatatttgaatgtatttagaaaaataaacaaataggggttccgcgcacatttccccgaaaagtgccacctgacgttaactataacggtcctaaggtagcgaaagctcagatctggatctcccgatcccctatggtcgactctcagtacaatctgctctgatgccgcatagttaagccagtatctgctccctgcttgtgtgttggaggtcgctgagtagtgcgcgagcaaaatttaagctacaacaaggcaaggcttgaccgacaattgcatgaagaatctgcttagggttaggcgttttgcgctgcttcgcgatgtacgggccagatatacgcgttgacattgattattgactagttattaatagtaatcaattacggggtcattagttcatagcccatatatggagttccgcgttacataacttacggtaaatggcccgcctggctgaccgcccaacgacccccgcccattgacgtcaataatgacgtatgttcccatagtaacgccaatagggactttccattgacgtcaatgggtggagtatttacggtaaactgcccacttggcagtacatcaagtgtatcatatgccaagtacgccccctattgacgtcaatgacggtaaatggcccgcctggcattatgcccagtacatgaccttatgggactttcctacttggcagtacatctacgtattagtcatcgctattaccatggtgatgcggttttggcagtacatcaatgggcgtggatagcggtttgactcacggggatttccaagtctccaccccattgacgtcaatgggagtttgttttggaaccaaaatcaacgggactttccaaaatgtcgtaacaactccgccccattgacgcaaatgggcggtaggcgtgtacggtgggaggtctatataagcagagctctccctatcagtgatagagatctccctatcagtgatagagatcgtcgacgagctcgtttagtgaaccgtcagatcgcctggagacgccatccacgctgttttgacctccatagagctagcgatatcaacaagtttgtacaaaaaagttggcgtttaaaccgctgatcagcctcgactgtgccttctagttgccagccatctgttgtttgcccctcccccgtgccttccttgaccctggaaggtgccactcccactgtcctttcctaataaaatgaggaaattgcatcgcattgtctgagtaggtgtcattctattctggggggtggggtggggcaggacagcaagggggaggattgggaagacaatagcaggcatgctggggatgcggtgggctctatggcttctgaggcggaaagaaccagcagatcgatctgcatctatgtcgggtgcggagaaagaggtaatgaaatggcattatgggtattatgggtctgcattaatgaatcggccaacggatccatatgcggtgtgaaataccgcacagatgcgtaaggagaaaataccgcatcaggcgctcttccgcttcctcgctcactgactcgctgcgctcggtcgttcggctgcggcgagcggtatcagctcactcaaaggcggtaatacggttatccacagaatcaggggataacgcaggaaagaacatgtgagcaaaaggccagcaaaaggccaggaaccgtaaaaaggccgcgttgctggcgtttttccataggctccgcccccctgacgagcatcacaaaaatcgacgctcaagtcagaggtggcgaaacccgacaggactataaagataccaggcgtttccccctggaagctccctcgtgcgctctcctgttccgaccctgccgcttaccggatacctgtccgcctttctcccttcgggaagcgtggcgctttctcatagctcacgctgtaggtatctcagttcggtgtaggtcgttcgctccaagctgggctgtgtgcacgaaccccccgttcagcccgaccgctgcgccttatccggtaactatcgtcttgagtccaacccggtaagacacgacttatcgccactggcagcagccactggtaacaggattagcagagcgaggtatgtaggcggtgctacagagttcttgaagtggtggcctaactacggctacactagaaggacagtatttggtatctgcgctctgctgaagccagttaccttcggaaaaagagttggtagctcttgatccggcaaacaaaccaccgctggtagcggtggtttttttgtttgcaagcagcagattacgcgcagaaaaaaaggatctcaagaagatcctttgatcttttctacggggtctgacgctcagtggaacgaaaactcacgttaagggattttggtcatgagattatcaaaaaggatcttcacctagatccttttaaattaaaaatgaagttttaaatcaatctaaagtatatatgagtaaacttggtctgacagttaccaatgcttaatcagtgaggcacctatctcagcgatctgtctatttcgttcatccatagttgcctgactccccgtcgtgtagataactacgatacgggagggcttaccatctggccccagtgctgcaatgataccgcgagacccacgctcaccggctccagatttatcagcaataaaccagccagccggaagggccgagcgcagaagtggtcctgcaactttatccgcctccatccagtctattaattgttgccgggaagctagagtaagtagttcgccagttaatagtttgcgcaacgttgttgaaaaaggatcttcacctagatccttttcacgtagaaagccagtccgcagaaacggtgctgaccccggatgaatgtcagctactgggctatctggacaagggaaaacgcaagcgcaaagagaaagcaggtagcttgcagtgggcttacatggcgatagctagactgggcggttttatggacagcaagcgaaccggaattgccagctggggcgccctctggtaaggttgggaagccctgcaaagtaaactggatggctttctcgccgccaaggatctgatggcgcaggggatcaagctctgatcaagagacaggatgaggatcgtttcgcatgattgaacaagatggattgcacgcaggttctccggccgcttgggtggagaggctattcggctatgactgggcacaacagacaatcggctgctctgatgccgccgtgttccggctgtcagcgcaggggcgcccggttctttttgtcaagaccgacctgtccggtgccctgaatgaactgcaagacgaggcagcgcggctatcgtggctggccacgacgggcgttccttgcgcagctgtgctcgacgttgtcactgaagcgggaagggactggctgctattgggcgaagtgccggggcaggatctcctgtcatctcaccttgctcctgccgagaaagtatccatcatggctgatgcaatgcggcggctgcatacgcttgatccggctacctgcccattcgaccaccaagcgaaacatcgcatcgagcgagcacgtactcggatggaagccggtcttgtcgatcaggatgatctggacgaagagcatcaggggctcgcgccagccgaactgttcgccaggctcaaggcgagcatgcccgacggcgaggatctcgtcgtgacccatggcgatgcctgcttgccgaatatcatggtggaaaatggccgcttttctggattcatcgactgtggccggctgggtgtggcggaccgctatcaggacatagcgttggctacccgtgatattgctgaagagcttggcggcgaatgggctgaccgcttcctcgtgctttacggtatcgccgctcccgattcgcagcgcatcgccttctatcgccttcttgacgagttcttctgaattttgttaaaatttttgttaaatcagctcattttttaaccaataggccgaaatcggcaacatcccttataaatcaaaagaatagaccgcgatagggttgagtgttgttccagtttggaacaagagtccactattaaagaacgtggactccaacgtcaaagggcgaaaaaccgtctatcagggcgatggcccactacgtgaaccatcacccaaatcaagttttttgcggtcgaggtgccgtaaagctctaaatcggaaccctaaagggagcccccgatttagagcttgacggggaaagccggcgaacgtggcgagaaaggaagggaagaaagcgaaaggagcgggcgctagggcgctggcaagtgtagcggtcacgctgcgcgtaaccaccacacccgcgcgcttaatgcgccgctacagggcgcgtccattcgccattcaggatcgaattaattcttaattaacatcatcaataatatacctt

SEQ ID NO: 12 - DNA, 24 bp, Artificial Sequence
  FLAG tag
gactacaaagacgatgacgacaag

SEQ ID NO: 13 - DNA, 18 bp, Artificial Sequence
  6X His tag
catcatcaccatcaccat

SEQ ID NO: 14 - DNA, 51 bp, Artificial Sequence
  Signal peptide
atgtggaccctggtgagctgggtggccttaacagcagggctggtggctgga